European Patent Specification EP 3 778 874 B1, published January 28, 2026. Title: Composition for inducing de-differentiation from somatic cell into induced pluripotent stem cell and method for inducing de-differentiation using the same. Applicant: Industry-University Cooperation Foundation Korea University. The sequence listing filed with the application follows.

SEQUENCE LISTING (7 sequences)

SEQ ID NO: 1 - DNA, 18 bp, Artificial Sequence
  Artificial sequences
ctggccgtggctctcttg

SEQ ID NO: 2 - DNA, 20 bp, Artificial Sequence
  Artificial sequences
ccttggcaaaactgcacctt

SEQ ID NO: 3 - DNA, 57 bp, shRNA lentiviral particles
gatccgtctactcatccaatgttattcaagagataacattggatgagtagacttttt

SEQ ID NO: 4 - DNA, 57 bp, shRNA lentiviral particles
gatcccctcaagattctagctatattcaagagatatagctagaatcttgaggttttt

SEQ ID NO: 5 - DNA, 57 bp, shRNA lentiviral particles
gatccgccactaaattgacacttattcaagagataagtgtcaatttagtggcttttt

SEQ ID NO: 6 - DNA, 23 bp, Artificial Sequence
  Artificial sequences
caatgaatgaatgaatggctaag

SEQ ID NO: 7 - DNA, 25 bp, Artificial Sequence
  Artificial sequences
aaagttttcaaggttcgtccgtgtt